European Patent Application EP 4 596 579 A1, published August 6, 2025. Title: 能够识别ANG-2的抗体或抗原结合片段和同时识别VEGF和ANG-2的双抗. Applicant: 科兴生物制药股份有限公司. Application CN. The sequence listing filed with the application follows.

SEQUENCE LISTING (40 sequences)

SEQ ID NO: 1 - protein, 5 aa, synthetic construct
YYSIG

SEQ ID NO: 2 - protein, 17 aa, synthetic construct
CISRTDGSTYYADSVKG

SEQ ID NO: 3 - protein, 18 aa, synthetic construct
KGARYSGSYLCGLDEYDY

SEQ ID NO: 4 - protein, 5 aa, synthetic construct
SATMS

SEQ ID NO: 5 - protein, 17 aa, synthetic construct
LIAYAGGSTTYADSVKG

SEQ ID NO: 6 - protein, 7 aa, synthetic construct
RRYNRDF

SEQ ID NO: 7 - protein, 5 aa, synthetic construct
YYAIG

SEQ ID NO: 8 - protein, 17 aa, synthetic construct
CISSGDGSTYYADSVKG

SEQ ID NO: 9 - protein, 23 aa, synthetic construct
VRSGSKCLVTRGTVVAAGQLYEY

SEQ ID NO: 10 - protein, 5 aa, synthetic construct
FSTVR

SEQ ID NO: 11 - protein, 16 aa, synthetic construct
TLLDDGSTNYADSVKG

SEQ ID NO: 12 - protein, 12 aa, synthetic construct
DGRTGWGPRGDY

SEQ ID NO: 13 - protein, 15 aa, synthetic construct
THDDGSTNYEDSVKG

SEQ ID NO: 14 - protein, 12 aa, synthetic construct
DGSTGWGPRGDY

SEQ ID NO: 15 - DNA, 1293 bp, synthetic construct
  source 1..1293: mol_type = other DNA
tccgatacaggaaggccttttgtggaaatgtactccgagatccccgagatcatccacatgaccgagggcagggaactggtgattccttgcagggtgacctcccccaatatcaccgtgaccctgaagaagttccccctggacaccctgatccccgacggaaaaaggatcatctgggactccaggaagggcttcatcatctccaacgccacctacaaggagatcggcctgctgacctgtgaggccacagtgaatggccatctgtataagaccaactacctgacccacaggcagaccaacaccatcatcgacgtggtgctgtccccctcccatggcattgagctgtctgttggcgagaaactggtgctgaactgtaccgctaggaccgaactgaatgtgggcatcgactttaactgggagtacccctcctccaagcaccagcacaaaaagctggtgaacagggacctgaagacccagtccggctccgaaatgaaaaagttcctgtccaccctgaccatcgacggcgtgacaaggtccgatcaaggcctgtatacctgtgctgcctcctccggcctgatgaccaaaaagaactccaccttcgtgagggtgcacgagaaggacaagacccacacctgccccccttgtcccgctcctgaactgctgggaggaccttctgtgtttctgtttccccctaaacccaaagataccctgatgatctccaggacccccgaggtgacatgtgtggtggttgatgtgtcccatgaagaccccgaggtgaagttcaactggtacgtggacggcgtggaggtgcacaatgctaagaccaagcccagggaggagcagtataactccacctacagggtggtgtccgtgctgaccgtgctgcatcaagactggctgaacggcaaggagtataagtgcaaggtgtccaacaaggccctgcccgcccctattgaaaagaccatttccaaggccaagggccagcccagggagcctcaagtttatacactgcctccctccagggacgagctgacaaaaaatcaggtgtccctgacctgcctggtgaagggcttttacccctccgacatcgccgtggagtgggaatccaatggccagcccgaaaacaactacaagaccaccccccccgtgctggactccgacgggtccttttttctgtactccaagctgaccgtggacaagtccaggtggcagcagggaaatgtgttctcctgctccgtgatgcacgaggccctgcataaccactacacccagaagtccctgtccctgtcccccgga

SEQ ID NO: 16 - protein, 127 aa, synthetic construct
QLQLVESGGGLVQPGGSLRLSCAASGFTLGYYSIGWFRQAPGKEREGVSCISRTDGSTYYADSVKGRFTISRDNAKNTVYLQMNNLKPEDTAVYYCAVKGARYSGSYLCGLDEYDYWGQGTQVTVSS

SEQ ID NO: 17 - protein, 116 aa, synthetic construct
QVQLVESGGGLVQPGGSLRLSCAASGFSFSSATMSWHRQTPGKERTMVALIAYAGGSTTYADSVKGRFTISRDNAKNTVYLQMSNLKPEDTAVYYCNTRRYNRDFWGQGTQVTVSS

SEQ ID NO: 18 - protein, 132 aa, synthetic construct
QLQLVESGGGLVQPGGSLRLSCAASGFTLDYYAIGWFRQVPGKAREGLSCISSGDGSTYYADSVKGRFTISRDNTKNTVYLQMNSLKPEDTAVYSCAAVRSGSKCLVTRGTVVAAGQLYEYWGQGTQVTVSS

SEQ ID NO: 19 - protein, 120 aa, synthetic construct
QVQLVESGGGLVQPGGSLRLSCAASGSIFSFSTVRWYRQAPGKQREPVATLLDDGSTNYADSVKGRFTISTDNAKNTVYLQMNSLKPEDTAVYYCNADGRTGWGPRGDYWGRGTQVTVSS

SEQ ID NO: 20 - protein, 119 aa, synthetic construct
QVQLVESGGGLVQPGGSLRLSCAASGSSFKFSTVRWYRQAPGKQREPVATHDDGSTNYEDSVKGRFTISRDNAKNTAFLQMNSLKPEDTAVYYCNADGSTGWGPRGDYWGRGTQVTVSS

SEQ ID NO: 21 - protein, 359 aa, synthetic construct
QLQLVESGGGLVQPGGSLRLSCAASGFTLGYYSIGWFRQAPGKEREGVSCISRTDGSTYYADSVKGRFTISRDNAKNTVYLQMNNLKPEDTAVYYCAVKGARYSGSYLCGLDEYDYWGQGTQVTVSSEPKSADKTHTCPPCPAPELLGGPSVFLFPPKPKDTLMISRTPEVTCVVVDVSHEDPEVKFNWYVDGVEVHNAKTKPREEQYNSTYRVVSVLTVLHQDWLNGKEYKCKVSNKALPAPIEKTISKAKGQPREPQVYTLPPSREEMTKNQVSLTCLVKGFYPSDIAVEWESNGQPENNYKTTPPVLDSDGSFFLYSKLTVDKSRWQQGNVFSCSVMHEALHNHYTQKSLSLSPGK

SEQ ID NO: 22 - protein, 348 aa, synthetic construct
QVQLVESGGGLVQPGGSLRLSCAASGFSFSSATMSWHRQTPGKERTMVALIAYAGGSTTYADSVKGRFTISRDNAKNTVYLQMSNLKPEDTAVYYCNTRRYNRDFWGQGTQVTVSSEPKSADKTHTCPPCPAPELLGGPSVFLFPPKPKDTLMISRTPEVTCVVVDVSHEDPEVKFNWYVDGVEVHNAKTKPREEQYNSTYRVVSVLTVLHQDWLNGKEYKCKVSNKALPAPIEKTISKAKGQPREPQVYTLPPSREEMTKNQVSLTCLVKGFYPSDIAVEWESNGQPENNYKTTPPVLDSDGSFFLYSKLTVDKSRWQQGNVFSCSVMHEALHNHYTQKSLSLSPGK

SEQ ID NO: 23 - protein, 364 aa, synthetic construct
QLQLVESGGGLVQPGGSLRLSCAASGFTLDYYAIGWFRQVPGKAREGLSCISSGDGSTYYADSVKGRFTISRDNTKNTVYLQMNSLKPEDTAVYSCAAVRSGSKCLVTRGTVVAAGQLYEYWGQGTQVTVSSEPKSADKTHTCPPCPAPELLGGPSVFLFPPKPKDTLMISRTPEVTCVVVDVSHEDPEVKFNWYVDGVEVHNAKTKPREEQYNSTYRVVSVLTVLHQDWLNGKEYKCKVSNKALPAPIEKTISKAKGQPREPQVYTLPPSREEMTKNQVSLTCLVKGFYPSDIAVEWESNGQPENNYKTTPPVLDSDGSFFLYSKLTVDKSRWQQGNVFSCSVMHEALHNHYTQKSLSLSPGK

SEQ ID NO: 24 - protein, 352 aa, synthetic construct
QVQLVESGGGLVQPGGSLRLSCAASGSIFSFSTVRWYRQAPGKQREPVATLLDDGSTNYADSVKGRFTISTDNAKNTVYLQMNSLKPEDTAVYYCNADGRTGWGPRGDYWGRGTQVTVSSEPKSADKTHTCPPCPAPELLGGPSVFLFPPKPKDTLMISRTPEVTCVVVDVSHEDPEVKFNWYVDGVEVHNAKTKPREEQYNSTYRVVSVLTVLHQDWLNGKEYKCKVSNKALPAPIEKTISKAKGQPREPQVYTLPPSREEMTKNQVSLTCLVKGFYPSDIAVEWESNGQPENNYKTTPPVLDSDGSFFLYSKLTVDKSRWQQGNVFSCSVMHEALHNHYTQKSLSLSPGK

SEQ ID NO: 25 - protein, 351 aa, synthetic construct
QVQLVESGGGLVQPGGSLRLSCAASGSSFKFSTVRWYRQAPGKQREPVATHDDGSTNYEDSVKGRFTISRDNAKNTAFLQMNSLKPEDTAVYYCNADGSTGWGPRGDYWGRGTQVTVSSEPKSADKTHTCPPCPAPELLGGPSVFLFPPKPKDTLMISRTPEVTCVVVDVSHEDPEVKFNWYVDGVEVHNAKTKPREEQYNSTYRVVSVLTVLHQDWLNGKEYKCKVSNKALPAPIEKTISKAKGQPREPQVYTLPPSREEMTKNQVSLTCLVKGFYPSDIAVEWESNGQPENNYKTTPPVLDSDGSFFLYSKLTVDKSRWQQGNVFSCSVMHEALHNHYTQKSLSLSPGK

SEQ ID NO: 26 - protein, 431 aa, synthetic construct
SDTGRPFVEMYSEIPEIIHMTEGRELVIPCRVTSPNITVTLKKFPLDTLIPDGKRIIWDSRKGFIISNATYKEIGLLTCEATVNGHLYKTNYLTHRQTNTIIDVVLSPSHGIELSVGEKLVLNCTARTELNVGIDFNWEYPSSKHQHKKLVNRDLKTQSGSEMKKFLSTLTIDGVTRSDQGLYTCAASSGLMTKKNSTFVRVHEKDKTHTCPPCPAPELLGGPSVFLFPPKPKDTLMISRTPEVTCVVVDVSHEDPEVKFNWYVDGVEVHNAKTKPREEQYNSTYRVVSVLTVLHQDWLNGKEYKCKVSNKALPAPIEKTISKAKGQPREPQVYTLPPSRDELTKNQVSLTCLVKGFYPSDIAVEWESNGQPENNYKTTPPVLDSDGSFFLYSKLTVDKSRWQQGNVFSCSVMHEALHNHYTQKSLSLSPG

SEQ ID NO: 27 - protein, 20 aa, synthetic construct
GGGGSGGGGSGGGGSGGGGS

SEQ ID NO: 28 - protein, 578 aa, synthetic construct
SDTGRPFVEMYSEIPEIIHMTEGRELVIPCRVTSPNITVTLKKFPLDTLIPDGKRIIWDSRKGFIISNATYKEIGLLTCEATVNGHLYKTNYLTHRQTNTIIDVVLSPSHGIELSVGEKLVLNCTARTELNVGIDFNWEYPSSKHQHKKLVNRDLKTQSGSEMKKFLSTLTIDGVTRSDQGLYTCAASSGLMTKKNSTFVRVHEKDKTHTCPPCPAPELLGGPSVFLFPPKPKDTLMISRTPEVTCVVVDVSHEDPEVKFNWYVDGVEVHNAKTKPREEQYNSTYRVVSVLTVLHQDWLNGKEYKCKVSNKALPAPIEKTISKAKGQPREPQVYTLPPSRDELTKNQVSLTCLVKGFYPSDIAVEWESNGQPENNYKTTPPVLDSDGSFFLYSKLTVDKSRWQQGNVFSCSVMHEALHNHYTQKSLSLSPGGGGGSGGGGSGGGGSGGGGSQLQLVESGGGLVQPGGSLRLSCAASGFTLGYYSIGWFRQAPGKEREGVSCISRTDGSTYYADSVKGRFTISRDNAKNTVYLQMNNLKPEDTAVYYCAVKGARYSGSYLCGLDEYDYWGQGTQVTVSS

SEQ ID NO: 29 - protein, 567 aa, synthetic construct
SDTGRPFVEMYSEIPEIIHMTEGRELVIPCRVTSPNITVTLKKFPLDTLIPDGKRIIWDSRKGFIISNATYKEIGLLTCEATVNGHLYKTNYLTHRQTNTIIDVVLSPSHGIELSVGEKLVLNCTARTELNVGIDFNWEYPSSKHQHKKLVNRDLKTQSGSEMKKFLSTLTIDGVTRSDQGLYTCAASSGLMTKKNSTFVRVHEKDKTHTCPPCPAPELLGGPSVFLFPPKPKDTLMISRTPEVTCVVVDVSHEDPEVKFNWYVDGVEVHNAKTKPREEQYNSTYRVVSVLTVLHQDWLNGKEYKCKVSNKALPAPIEKTISKAKGQPREPQVYTLPPSRDELTKNQVSLTCLVKGFYPSDIAVEWESNGQPENNYKTTPPVLDSDGSFFLYSKLTVDKSRWQQGNVFSCSVMHEALHNHYTQKSLSLSPGGGGGSGGGGSGGGGSGGGGSQVQLVESGGGLVQPGGSLRLSCAASGFSFSSATMSWHRQTPGKERTMVALIAYAGGSTTYADSVKGRFTISRDNAKNTVYLQMSNLKPEDTAVYYCNTRRYNRDFWGQGTQVTVSS

SEQ ID NO: 30 - protein, 583 aa, synthetic construct
SDTGRPFVEMYSEIPEIIHMTEGRELVIPCRVTSPNITVTLKKFPLDTLIPDGKRIIWDSRKGFIISNATYKEIGLLTCEATVNGHLYKTNYLTHRQTNTIIDVVLSPSHGIELSVGEKLVLNCTARTELNVGIDFNWEYPSSKHQHKKLVNRDLKTQSGSEMKKFLSTLTIDGVTRSDQGLYTCAASSGLMTKKNSTFVRVHEKDKTHTCPPCPAPELLGGPSVFLFPPKPKDTLMISRTPEVTCVVVDVSHEDPEVKFNWYVDGVEVHNAKTKPREEQYNSTYRVVSVLTVLHQDWLNGKEYKCKVSNKALPAPIEKTISKAKGQPREPQVYTLPPSRDELTKNQVSLTCLVKGFYPSDIAVEWESNGQPENNYKTTPPVLDSDGSFFLYSKLTVDKSRWQQGNVFSCSVMHEALHNHYTQKSLSLSPGGGGGSGGGGSGGGGSGGGGSQLQLVESGGGLVQPGGSLRLSCAASGFTLDYYAIGWFRQVPGKAREGLSCISSGDGSTYYADSVKGRFTISRDNTKNTVYLQMNSLKPEDTAVYSCAAVRSGSKCLVTRGTVVAAGQLYEYWGQGTQVTVSS

SEQ ID NO: 31 - protein, 571 aa, synthetic construct
SDTGRPFVEMYSEIPEIIHMTEGRELVIPCRVTSPNITVTLKKFPLDTLIPDGKRIIWDSRKGFIISNATYKEIGLLTCEATVNGHLYKTNYLTHRQTNTIIDVVLSPSHGIELSVGEKLVLNCTARTELNVGIDFNWEYPSSKHQHKKLVNRDLKTQSGSEMKKFLSTLTIDGVTRSDQGLYTCAASSGLMTKKNSTFVRVHEKDKTHTCPPCPAPELLGGPSVFLFPPKPKDTLMISRTPEVTCVVVDVSHEDPEVKFNWYVDGVEVHNAKTKPREEQYNSTYRVVSVLTVLHQDWLNGKEYKCKVSNKALPAPIEKTISKAKGQPREPQVYTLPPSRDELTKNQVSLTCLVKGFYPSDIAVEWESNGQPENNYKTTPPVLDSDGSFFLYSKLTVDKSRWQQGNVFSCSVMHEALHNHYTQKSLSLSPGGGGGSGGGGSGGGGSGGGGSQVQLVESGGGLVQPGGSLRLSCAASGSIFSFSTVRWYRQAPGKQREPVATLLDDGSTNYADSVKGRFTISTDNAKNTVYLQMNSLKPEDTAVYYCNADGRTGWGPRGDYWGRGTQVTVSS

SEQ ID NO: 32 - protein, 570 aa, synthetic construct
SDTGRPFVEMYSEIPEIIHMTEGRELVIPCRVTSPNITVTLKKFPLDTLIPDGKRIIWDSRKGFIISNATYKEIGLLTCEATVNGHLYKTNYLTHRQTNTIIDVVLSPSHGIELSVGEKLVLNCTARTELNVGIDFNWEYPSSKHQHKKLVNRDLKTQSGSEMKKFLSTLTIDGVTRSDQGLYTCAASSGLMTKKNSTFVRVHEKDKTHTCPPCPAPELLGGPSVFLFPPKPKDTLMISRTPEVTCVVVDVSHEDPEVKFNWYVDGVEVHNAKTKPREEQYNSTYRVVSVLTVLHQDWLNGKEYKCKVSNKALPAPIEKTISKAKGQPREPQVYTLPPSRDELTKNQVSLTCLVKGFYPSDIAVEWESNGQPENNYKTTPPVLDSDGSFFLYSKLTVDKSRWQQGNVFSCSVMHEALHNHYTQKSLSLSPGGGGGSGGGGSGGGGSGGGGSQVQLVESGGGLVQPGGSLRLSCAASGSSFKFSTVRWYRQAPGKQREPVATHDDGSTNYEDSVKGRFTISRDNAKNTAFLQMNSLKPEDTAVYYCNADGSTGWGPRGDYWGRGTQVTVSS

SEQ ID NO: 33 - DNA, 381 bp, synthetic construct
  source 1..381: mol_type = other DNA
cagctgcagctggtggagtccggaggaggactggtgcagcctggaggaagcctgaggctgtcctgcgctgcttccggatttaccctgggatattactctattggctggttcaggcaggcccccggaaaagagagagagggagtgtcttgcatttcccgcacagacggaagcacctactacgctgactccgtcaagggcaggttcacaatctcccgcgacaatgccaagaacacagtgtacctgcagatgaacaacctgaagcccgaggacaccgccgtgtattactgcgctgtgaagggcgctaggtatagcggaagctacctgtgcggcctggacgagtatgactactggggacagggcacccaggtcaccgtgtcctcc

SEQ ID NO: 34 - DNA, 348 bp, synthetic construct
  source 1..348: mol_type = other DNA
caggtgcagctggtggagtccggaggaggactggtgcagcctggaggaagcctgaggctgtcctgcgctgcttccggatttagttttagtagtgcaacaatgtcctggcacaggcagacccctggaaaagagaggacaatggttgctctgattgcctacgccggaggatctacaacctacgctgattcagtgaagggccggttcaccatctccagagacaacgctaagaacaccgtgtacctgcagatgagcaacctgaagcctgaagatactgctgtgtattactgcaacaccaggaggtacaacagggacttttggggccagggcacccaggtgaccgtgtcctcc

SEQ ID NO: 35 - DNA, 396 bp, synthetic construct
  source 1..396: mol_type = other DNA
cagctgcagctggtggagtccggaggaggactggtgcagcctggaggaagcctgaggctgtcctgcgctgcttccggatttaccctggactattatgccattggctggttccggcaggtccctggaaaagctagagagggactgagctgcatttcctctggagacgggtccacctactacgctgattctgtgaagggcagatttaccatctcccgggacaatactaagaacaccgtgtacctgcagatgaacagcctgaaacccgaggacaccgccgtgtattcctgcgctgctgtgagatccggctctaagtgtctggtgaccaggggtaccgtggtggctgctggacagctgtatgaatactggggccagggcacacaggtgacagtgtcctcc

SEQ ID NO: 36 - DNA, 360 bp, synthetic construct
  source 1..360: mol_type = other DNA
caggtgcagctggtggagtccggaggaggactggtgcagcctggaggaagcctgaggctgtcctgcgctgcttccggaagcatttttagttttagtaccgtgaggtggtacaggcaggctcctggaaaacagagggagcctgtggctactctgctggatgacggttccaccaactacgccgactccgtgaagggaaggttcaccatctccaccgacaacgccaagaacacagtctatctgcagatgaacagcctgaaacccgaagatactgctgtgtactactgcaacgccgacggaaggaccggatggggacctaggggagactattggggaaggggaacccaggtgaccgtgtcctcc

SEQ ID NO: 37 - DNA, 357 bp, synthetic construct
  source 1..357: mol_type = other DNA
caggtgcagctggtggagtccggaggaggactggtgcagcctggaggaagcctgaggctgtcctgcgctgcttccggaagctcctttaaattttccacagtcaggtggtacaggcaggcccctggaaaacagagggagcctgtggctactcatgacgacggatctaccaactacgaggactccgtgaaaggcaggttcacaatcagcagggacaacgccaagaacaccgcattcctgcagatgaacagcctgaagcctgaggataccgccgtgtactactgcaacgccgacggatctaccgggtggggacctaggggagactattggggaaggggaacccaggtgaccgtctcctcc

SEQ ID NO: 38 - protein, 232 aa, synthetic construct
EPKSADKTHTCPPCPAPELLGGPSVFLFPPKPKDTLMISRTPEVTCVVVDVSHEDPEVKFNWYVDGVEVHNAKTKPREEQYNSTYRVVSVLTVLHQDWLNGKEYKCKVSNKALPAPIEKTISKAKGQPREPQVYTLPPSREEMTKNQVSLTCLVKGFYPSDIAVEWESNGQPENNYKTTPPVLDSDGSFFLYSKLTVDKSRWQQGNVFSCSVMHEALHNHYTQKSLSLSPGK

SEQ ID NO: 39 - DNA, 696 bp, synthetic construct
  source 1..696: mol_type = other DNA
gagcccaaatctgctgacaaaactcacacatgcccaccgtgcccagcacctgaactcctggggggaccgtcagtcttcctcttccccccaaaacccaaggacaccctcatgatctcccggacccccgaggtcacatgcgtggtggtggacgtgagccacgaagaccctgaggtcaagttcaactggtacgtggacggcgtggaggtgcataatgccaagacaaagccgcgggaggagcagtacaacagcacgtaccgtgtggtcagcgtcctcaccgtcctgcaccaggactggctgaatggcaaggagtacaagtgcaaggtctccaacaaagccctcccagcccccatcgagaaaaccatctccaaagccaaagggcagccccgagaaccacaggtgtacaccctgcccccatcccgggaggagatgaccaagaaccaggtcagcctgacctgcctggtcaaaggcttctatcccagcgacatcgccgtggagtgggagagcaatgggcagccggagaacaactacaagaccacgcctcccgtgctggactccgacggctccttcttcctctacagcaagctcaccgtggacaagagcaggtggcagcaggggaacgtcttctcatgctccgtgatgcatgaggctctgcacaaccactacacgcagaagagcctctccctgtctccgggtaaa

SEQ ID NO: 40 - DNA, 60 bp, synthetic construct
  source 1..60: mol_type = other DNA
ggaggaggaggatctggaggaggagggtccggaggaggaggaagcggaggaggaggaagc